European Patent Application EP 4 563 698 A1, published June 4, 2025. Title: ENZYME ELECTRODE, REDUCTION DEVICE, REDUCTION METHOD, MODIFIED PROTEIN, AND MODIFIED PROTEIN MANUFACTURING METHOD. Applicant: Panasonic Intellectual Property Management Co., Ltd. Application WO. The sequence listing filed with the application follows.

SEQUENCE LISTING (18 sequences)

SEQ ID NO: 1 - DNA, 348 bp, synthetic construct
  source 1..348: mol_type = other DNA
atggcgaaaacggaaccgtcggagaaatcagtagagattatgaggaaattctccgagcaatatgctcgtcgctctgggacttacttctgtgttgataaaggagttacttcagtcgttattaagggtttggctgagcataaagattcatatggtgcaccgctttgcccttgcagacactatgatgataaagctgctgaggttggacaaggcttttggaattgtccgtgtgttccaatgagagagaggaaggagtgccattgtatgcttttcttaactcctgataatgatttcgctggaaaagatcagacgattacatcggatgaaataaaagaaactacagctaacatg

SEQ ID NO: 2 - DNA, 333 bp, synthetic construct
  source 1..333: mol_type = other DNA
atggcagcaaagaagcaaactttcaactcttttgatgatttgttgcagaactctgataaacctgtacttgtagacttctatgctacttggtgtggtccatgtcagcttatggtacctatactcaatgaagtgagtgaaacactgaaagatataattgcagttgtgaaaattgatactgagaagtacccaagtcttgctaacaaataccagattgaggctttgcccacattcatcttattcaaagacggcaaactctgggaccgtttcgagggtgccttgccagcgaaccaactcgttgagcgtattgagaattctttgcaagtgaaacagtag

SEQ ID NO: 3 - DNA, 15 bp, synthetic construct
  source 1..15: mol_type = other DNA
ggcggcggcggcagc

SEQ ID NO: 4 - DNA, 30 bp, synthetic construct
  source 1..30: mol_type = other DNA
ggcggcggcggcagcggcggcggcggcagc

SEQ ID NO: 5 - DNA, 45 bp, synthetic construct
  source 1..45: mol_type = other DNA
ggcggcggcggcagcggcggcggcggcagcggcggcggcggcagc

SEQ ID NO: 6 - DNA, 339 bp, synthetic construct
  source 1..339: mol_type = other DNA
atggatattgctgtgaaatcggcggcttctgtagacgcggacgctgatctatcgtcatctacgtcgttggagacggaggaagacgagaaagcgaaggagaagattggagctagggttagggttacggttccgttgaaagtttaccatgtggttcgtgtaccggaggttgaattgatgggaatggaaggttttatcaaagattacgtcgttctttggaaaggaaagaaaatctcagctaatctgccgtttaaggtacagttcgtgaaagagatcgaaggtcgtggtcctgtcaaattcttcacgcatcttaaggaagacgagttcgagttaattgatccg

SEQ ID NO: 7 - DNA, 21 bp, synthetic construct
  source 1..21: mol_type = other DNA
caccaccaccaccaccactga

SEQ ID NO: 8 - DNA, 52 bp, synthetic construct
  source 1..52: mol_type = other DNA
ggagacggaggaagacgaggcagcggcggaggcgattggagctagggttagg

SEQ ID NO: 9 - DNA, 52 bp, synthetic construct
  source 1..52: mol_type = other DNA
cctaaccctagctccaatcgcctccgccgctgcctcgtcttcctccgtctcc

SEQ ID NO: 10 - DNA, 53 bp, synthetic construct
  source 1..53: mol_type = other DNA
tcctgtcaaattcttcacgcatcttcgtgaagacgagttcgagttaattgatc

SEQ ID NO: 11 - DNA, 53 bp, synthetic construct
  source 1..53: mol_type = other DNA
gatcaattaactcgaactcgtcttcacgaagatgcgtgaagaatttgacagga

SEQ ID NO: 12 - DNA, 45 bp, synthetic construct
  source 1..45: mol_type = other DNA
aagtacccaagtcttgctaaccgttaccagattgaggctttgccc

SEQ ID NO: 13 - DNA, 45 bp, synthetic construct
  source 1..45: mol_type = other DNA
gggcaaagcctcaatctggtaacggttagcaagacttgggtactt

SEQ ID NO: 14 - DNA, 59 bp, synthetic construct
  source 1..59: mol_type = other DNA
ttgaggctttgcccacattcatcttattccgtgacggccgtctctgggaccgtttcgag

SEQ ID NO: 15 - DNA, 59 bp, synthetic construct
  source 1..59: mol_type = other DNA
ctcgaaacggtcccagagacggccgtcacggaataagatgaatgtgggcaaagcctcaa

SEQ ID NO: 16 - protein, 241 aa, synthetic construct
MAKTEPSEKSVEIMRKFSEQYARRSGTYFCVDKGVTSVVIKGLAEHKDSYGAPLCPCRHYDDKAAEVGQGFWNCPCVPMRERKECHCMLFLTPDNDFAGKDQTITSDEIKETTANMGGGGSGGGGSGGGGSMAAKKQTFNSFDDLLQNSDKPVLVDFYATWCGPCQLMVPILNEVSETLKDIIAVVKIDTEKYPSLANRYQIEALPTFILFKDGKLWDRFEGALPANQLVERIENSLQVKQ

SEQ ID NO: 17 - protein, 241 aa, synthetic construct
MAKTEPSEKSVEIMRKFSEQYARRSGTYFCVDKGVTSVVIKGLAEHKDSYGAPLCPCRHYDDKAAEVGQGFWNCPCVPMRERKECHCMLFLTPDNDFAGKDQTITSDEIKETTANMGGGGSGGGGSGGGGSMAAKKQTFNSFDDLLQNSDKPVLVDFYATWCGPCQLMVPILNEVSETLKDIIAVVKIDTEKYPSLANRYQIEALPTFILFRDGRLWDRFEGALPANQLVERIENSLQVKQ

SEQ ID NO: 18 - protein, 119 aa, synthetic construct
MDIAVKSAASVDADADLSSSTSLETEEDERARERIGARVRVTVPLKVYHVVRVPEVELMGMEGFIKDYVVLWKGKKISANLPFKVQFVKEIEGRGPVKFFTHLREDEFELIDPHHHHHH